European Patent Application EP 4 556 484 A1, published May 21, 2025. Title: MODIFIED POLYPEPTIDE HAVING GLUCANASE ACTIVITY. Applicant: 씨제이제일제당 주식회사. The sequence listing filed with the application follows.

SEQUENCE LISTING (13 sequences)

SEQ ID NO: 1 - protein, 215 aa, synthetic construct
ATAVNTPFVADFNYHDSSQWEMSNWPNGEMFNCRWTPNNVKFENGKLKLTIDRDGSGYTCGEYRTKNYFGYGYYEVRMKPIKNPGVVSSFFTYTGPSDGTKWDEIDIEFLGYDTTKVQFNYYTNGQGGHEHIHYLGFDASQDFHTYGFFWARNSITWYVDGTAVYTATDNIPDTPGKIMMNAWNGIGVDDWLRPFNGRTNISAYYEYVKYYPNGN

SEQ ID NO: 2 - protein, 215 aa, synthetic construct
ATAVNTPFVADFNYHDSSQWEMSNWPNGEMFNCRWTPNNVKFENGKLKLTIDRDGSGYTCGEYRTKNYFGYGYYEVRMKPIKNPGVVSSFFTYTGPSDGTKWDEIDIEFLGYDTTKVQFNYYTNGQGGHEHIHYLGFDASQDFHTYGFFWARNSITWYVDGTAVYTATDNIPDTPGKIMMNAWNGIGVDDWLRPFNGRTPISAYYEYVKYYPNGN

SEQ ID NO: 3 - protein, 215 aa, synthetic construct
ATAVNTPFVADFNYHDSSQWEMSNWPNGEMFNCRWTPNNVKFENGKLKLTIDCDGSGYTCGEYRTKNYFGYGYYEVRMKPIKNPGVVSSFFTYTGPSDGTKWDEIDIEFLGYDTTKVQFNYYTNGQGGHEHIHYLGFDASQDFHTYGFFWARNSITWYVDGTAVYTATDNIPDTPGKIMMNAWNGIGVDDWLRPFNGRCNISAYYEYVKYYPNGN

SEQ ID NO: 4 - protein, 215 aa, synthetic construct
ATAVNTPFVADFNYHDSSQWEMSNWPNGEMFNCRWTPNNVKFENGKLKLTIDCDGSGYTCGEYRTKNYFGYGYYEVRMKPIKNPGVVSSFFTYTGPSDGTKWDEIDIEFLGYDTTKVQFNYYTNGQGGHEHIHYLGFDASQDFHTYGFFWARNSITWYVDGTAVYTATDNIPDTPGKIMMNAWNGIGVDDWLRPFNGRCPISAYYEYVKYYPNGN

SEQ ID NO: 5 - DNA, 645 bp, synthetic construct
  source 1..645: mol_type = other DNA
gctactgcggttaatacaccctttgtcgctgattttaactatcatgatagctctcagtgggaaatgtccaattggccgaacggcgagatgttcaactgccgttggaccccgaataacgttaaattcgagaacggcaagctcaagttgaccattgacagagatggcagcggttacacctgtggtgagtatcgtactaagaactatttcggctacggctactacgaggttcgtatgaaaccgattaaaaatccaggtgtagtgagctcgttcttcacgtacacgggtccgtctgatggcaccaaatgggacgaaatcgacatcgaatttctgggttatgataccaccaaggttcagtttaattattataccaacggtcagggtggtcatgaacatattcattatctgggttttgacgcaagccaagatttccacacctacggcttcttttgggcgcgtaacagcatcacctggtatgtggacggcaccgcggtgtataccgcgactgataacattccggataccccgggtaagatcatgatgaacgcgtggaacggaatcggtgtggatgactggctgcgcccttttaacggccgtaccaatattagcgcgtattacgagtacgttaagtattacccgaatggcaac

SEQ ID NO: 6 - DNA, 27 bp, synthetic construct
  source 1..27: mol_type = other DNA
aacggccgtaccccgattagcgcgtat

SEQ ID NO: 7 - DNA, 27 bp, synthetic construct
  source 1..27: mol_type = other DNA
atacgcgctaatcggggtacggccgtt

SEQ ID NO: 8 - DNA, 27 bp, synthetic construct
  source 1..27: mol_type = other DNA
ttgaccattgactgcgatggcagcggt

SEQ ID NO: 9 - DNA, 27 bp, synthetic construct
  source 1..27: mol_type = other DNA
tttaacggccgttgcaatattagcgcg

SEQ ID NO: 10 - DNA, 27 bp, synthetic construct
  source 1..27: mol_type = other DNA
accgctgccatcgcagtcaatggtcaa

SEQ ID NO: 11 - DNA, 27 bp, synthetic construct
  source 1..27: mol_type = other DNA
cgcgctaatattgcaacggccgttaaa

SEQ ID NO: 12 - DNA, 27 bp, synthetic construct
  source 1..27: mol_type = other DNA
aacggccgttgcccgattagcgcgtat

SEQ ID NO: 13 - DNA, 27 bp, synthetic construct
  source 1..27: mol_type = other DNA
atacgcgctaatcgggcaacggccgtt